European Patent Specification EP 4 048 798 B1, published June 26, 2024. Title: Adenovirus comprising a modified adenovirus hexon protein. Applicant: Universität Ulm. The sequence listing filed with the application follows.

SEQUENCE LISTING (53 sequences)

SEQ ID NO: 1 - protein, 20 aa, Human Adenovirus Species C
DEAATALEINLKKKKQAEQQ

SEQ ID NO: 2 - DNA, 2832 bp, Human Adenovirus Species C
atggctaccccttcgatgatgccgcagtggtcttacatgcacatctcgggccaggacgcctcggagtacctgagccccgggctggtgcagtttgcccgcgccaccgagacgtacttcagcctgaataacaagtttagaaaccccacggtggcgcctacgcacgacgtgaccacagaccggtcccagcgtttgacgctgcggttcatccctgtggaccgtgaggatactgcgtactcgtacaaggcgcggttcaccctagctgtgggtgataaccgtgtgctggacatggcttccacgtactttgacatccgcggcgtgctggacaggggccctacttttaagccctactctggcactgcctacaacgccctggctcccaagggtgccccaaatccttgcgaatgggatgaagctgctactgctcttgaaataaacctaaaaaagaaaaagcaagctgagcagcaaaaaactcacgtatttgggcaggcgccttattctggtataaatattacaaaggagggtattcaaataggtgtcgaaggtcaaacacctaaatatgccgataaaacatttcaacctgaacctcaaataggagaatctcagtggtacgaaacagaaattaatcatgcagctgggagagtcctaaaaaagactaccccaatgaaaccatgttacggttcatatgcaaaacccacaaatgaaaatggagggcaaggcattcttgtaaagcaacaaaatggaaagctagaaagtcaagtggaaatgcaatttttctcaactactgaggcagccgcaggcaatggtgataacttgactcctaaagtggtattgtacagtgaagatgtagatatagaaaccccagacactcatatttcttacatgcccactattaaggaaggtaactcacgagaactaatgggccaacaatctatgcccaacaggcctaattacattgcttttagggacaattttattggtctaatgtattacaacagcacgggtaatatgggtgttctggcgggccaagcatcgcagttgaatgctgttgtagatttgcaagacagaaacacagagctttcataccagcttttgcttgattccattggtgatagaaccaggtacttttctatgtggaatcaggctgttgacagctatgatccagatgttagaattattgaaaatcatggaactgaagatgaacttccaaattactgctttccactgggaggtgtgattaatacagagactcttaccaaggtaaaacctaaaacaggtcaggaaaatggatgggaaaaagatgctacagaattttcagataaaaatgaaataagagttggaaataattttgccatggaaatcaatctaaatgccaacctgtggagaaatttcctgtactccaacatagcgctgtatttgcccgacaagctaaagtacagtccttccaacgtaaaaatttctgataacccaaacacctacgactacatgaacaagcgagtggtggctcccgggctagtggactgctacattaaccttggagcacgctggtcccttgactatatggacaacgtcaacccatttaaccaccaccgcaatgctggcctgcgctaccgctcaatgttgctgggcaatggtcgctatgtgcccttccacatccaggtgcctcagaagttctttgccattaaaaacctccttctcctgccgggctcatacacctacgagtggaacttcaggaaggatgttaacatggttctgcagagctccctaggaaatgacctaagggttgacggagccagcattaagtttgatagcatttgcctttacgccaccttcttccccatggcccacaacaccgcctccacgcttgaggccatgcttagaaacgacaccaacgaccagtcctttaacgactatctctccgccgccaacatgctctaccctatacccgccaacgctaccaacgtgcccatatccatcccctcccgcaactgggcggctttccgcggctgggccttcacgcgccttaagactaaggaaaccccatcactgggctcgggctacgacccttattacacctactctggctctataccctacctagatggaaccttttacctcaaccacacctttaagaaggtggccattacctttgactcttctgtcagctggcctggcaatgaccgcctgcttacccccaacgagtttgaaattaagcgctcagttgacggggagggttacaacgttgcccagtgtaacatgaccaaagactggttcctggtacaaatgctagctaactataacattggctaccagggcttctatatcccagagagctacaaggaccgcatgtactccttctttagaaacttccagcccatgagccgtcaggtggtggatgatactaaatacaaggactaccaacaggtgggcatcctacaccaacacaacaactctggatttgttggctaccttgcccccaccatgcgcgaaggacaggcctaccctgctaacttcccctatccgcttataggcaagaccgcagttgacagcattacccagaaaaagtttctttgcgatcgcaccctttggcgcatcccattctccagtaactttatgtccatgggcgcactcacagacctgggccaaaaccttctctacgccaactccgcccacgcgctagacatgacttttgaggtggatcccatggacgagcccacccttctttatgttttgtttgaagtctttgacgtggtccgtgtgcaccagccgcaccgcggcgtcatcgaaaccgtgtacctgcgcacgcccttctcggccggcaacgccacaacataa

SEQ ID NO: 3 - protein, 943 aa, Human Adenovirus Species C
MATPSMMPQWSYMHISGQDASEYLSPGLVQFARATETYFSLNNKFRNPTVAPTHDVTTDRSQRLTLRFIPVDREDTAYSYKARFTLAVGDNRVLDMASTYFDIRGVLDRGPTFKPYSGTAYNALAPKGAPNPCEWDEAATALEINLKKKKQAEQQKTHVFGQAPYSGINITKEGIQIGVEGQTPKYADKTFQPEPQIGESQWYETEINHAAGRVLKKTTPMKPCYGSYAKPTNENGGQGILVKQQNGKLESQVEMQFFSTTEAAAGNGDNLTPKVVLYSEDVDIETPDTHISYMPTIKEGNSRELMGQQSMPNRPNYIAFRDNFIGLMYYNSTGNMGVLAGQASQLNAVVDLQDRNTELSYQLLLDSIGDRTRYFSMWNQAVDSYDPDVRIIENHGTEDELPNYCFPLGGVINTETLTKVKPKTGQENGWEKDATEFSDKNEIRVGNNFAMEINLNANLWRNFLYSNIALYLPDKLKYSPSNVKISDNPNTYDYMNKRVVAPGLVDCYINLGARWSLDYMDNVNPFNHHRNAGLRYRSMLLGNGRYVPFHIQVPQKFFAIKNLLLLPGSYTYEWNFRKDVNMVLQSSLGNDLRVDGASIKFDSICLYATFFPMAHNTASTLEAMLRNDTNDQSFNDYLSAANMLYPIPANATNVPISIPSRNWAAFRGWAFTRLKTKETPSLGSGYDPYYTYSGSIPYLDGTFYLNHTFKKVAITFDSSVSWPGNDRLLTPNEFEIKRSVDGEGYNVAQCNMTKDWFLVQMLANYNIGYQGFYIPESYKDRMYSFFRNFQPMSRQVVDDTKYKDYQQVGILHQHNNSGFVGYLAPTMREGQAYPANFPYPLIGKTAVDSITQKKFLCDRTLWRIPFSSNFMSMGALTDLGQNLLYANSAHALDMTFEVDPMDEPTLLYVLFEVFDVVRVHQPHRGVIETVYLRTPFSAGNATT

SEQ ID NO: 4 - DNA, 2859 bp, Human Adenovirus Species C
atggctaccccttcgatgatgccgcagtggtcttacatgcacatctcgggccaggacgcctcggagtacctgagccccgggctggtgcagtttgcccgcgccaccgagacgtacttcagcctgaataacaagtttagaaaccccacggtggcgcctacgcacgacgtgaccacagaccggtcccagcgtttgacgctgcggttcatccctgtggaccgtgaggatactgcgtactcgtacaaggcgcggttcaccctagctgtgggtgataaccgtgtgctggacatggcttccacgtactttgacatccgcggcgtgctggacaggggccctacttttaagccctactctggcactgcctacaacgccctggctcccaagggtgccccaaatccttgcgaatgggatgaagctgctactgctcttgaaataaacctagaagaagaggacgatgacaacgaagacgaagtagacgagcaagctgagcagcaaaaaactcacgtatttgggcaggcgccttattctggtataaatattacaaaggagggtattcaaataggtgtcgaaggtcaaacacctaaatatgccgataaaacatttcaacctgaacctcaaataggagaatctcagtggtacgaaacagaaattaatcatgcagctgggagagtcctaaaaaagactaccccaatgaaaccatgttacggttcatatgcaaaacccacaaatgaaaatggagggcaaggcattcttgtaaagcaacaaaatggaaagctagaaagtcaagtggaaatgcaatttttctcaactactgaggcagccgcaggcaatggtgataacttgactcctaaagtggtattgtacagtgaagatgtagatatagaaaccccagacactcatatttcttacatgcccactattaaggaaggtaactcacgagaactaatgggccaacaatctatgcccaacaggcctaattacattgcttttagggacaattttattggtctaatgtattacaacagcacgggtaatatgggtgttctggcgggccaagcatcgcagttgaatgctgttgtagatttgcaagacagaaacacagagctttcataccagcttttgcttgattccattggtgatagaaccaggtacttttctatgtggaatcaggctgttgacagctatgatccagatgttagaattattgaaaatcatggaactgaagatgaacttccaaattactgctttccactgggaggtgtgattaatacagagactcttaccaaggtaaaacctaaaacaggtcaggaaaatggatgggaaaaagatgctacagaattttcagataaaaatgaaataagagttggaaataattttgccatggaaatcaatctaaatgccaacctgtggagaaatttcctgtactccaacatagcgctgtatttgcccgacaagctaaagtacagtccttccaacgtaaaaatttctgataacccaaacacctacgactacatgaacaagcgagtggtggctcccgggctagtggactgctacattaaccttggagcacgctggtcccttgactatatggacaacgtcaacccatttaaccaccaccgcaatgctggcctgcgctaccgctcaatgttgctgggcaatggtcgctatgtgcccttccacatccaggtgcctcagaagttctttgccattaaaaacctccttctcctgccgggctcatacacctacgagtggaacttcaggaaggatgttaacatggttctgcagagctccctaggaaatgacctaagggttgacggagccagcattaagtttgatagcatttgcctttacgccaccttcttccccatggcccacaacaccgcctccacgcttgaggccatgcttagaaacgacaccaacgaccagtcctttaacgactatctctccgccgccaacatgctctaccctatacccgccaacgctaccaacgtgcccatatccatcccctcccgcaactgggcggctttccgcggctgggccttcacgcgccttaagactaaggaaaccccatcactgggctcgggctacgacccttattacacctactctggctctataccctacctagatggaaccttttacctcaaccacacctttaagaaggtggccattacctttgactcttctgtcagctggcctggcaatgaccgcctgcttacccccaacgagtttgaaattaagcgctcagttgacggggagggttacaacgttgcccagtgtaacatgaccaaagactggttcctggtacaaatgctagctaactataacattggctaccagggcttctatatcccagagagctacaaggaccgcatgtactccttctttagaaacttccagcccatgagccgtcaggtggtggatgatactaaatacaaggactaccaacaggtgggcatcctacaccaacacaacaactctggatttgttggctaccttgcccccaccatgcgcgaaggacaggcctaccctgctaacttcccctatccgcttataggcaagaccgcagttgacagcattacccagaaaaagtttctttgcgatcgcaccctttggcgcatcccattctccagtaactttatgtccatgggcgcactcacagacctgggccaaaaccttctctacgccaactccgcccacgcgctagacatgacttttgaggtggatcccatggacgagcccacccttctttatgttttgtttgaagtctttgacgtggtccgtgtgcaccagccgcaccgcggcgtcatcgaaaccgtgtacctgcgcacgcccttctcggccggcaacgccacaacataa

SEQ ID NO: 5 - protein, 952 aa, Human Adenovirus Species C
MATPSMMPQWSYMHISGQDASEYLSPGLVQFARATETYFSLNNKFRNPTVAPTHDVTTDRSQRLTLRFIPVDREDTAYSYKARFTLAVGDNRVLDMASTYFDIRGVLDRGPTFKPYSGTAYNALAPKGAPNPCEWDEAATALEINLEEEDDDNEDEVDEQAEQQKTHVFGQAPYSGINITKEGIQIGVEGQTPKYADKTFQPEPQIGESQWYETEINHAAGRVLKKTTPMKPCYGSYAKPTNENGGQGILVKQQNGKLESQVEMQFFSTTEAAAGNGDNLTPKVVLYSEDVDIETPDTHISYMPTIKEGNSRELMGQQSMPNRPNYIAFRDNFIGLMYYNSTGNMGVLAGQASQLNAVVDLQDRNTELSYQLLLDSIGDRTRYFSMWNQAVDSYDPDVRIIENHGTEDELPNYCFPLGGVINTETLTKVKPKTGQENGWEKDATEFSDKNEIRVGNNFAMEINLNANLWRNFLYSNIALYLPDKLKYSPSNVKISDNPNTYDYMNKRVVAPGLVDCYINLGARWSLDYMDNVNPFNHHRNAGLRYRSMLLGNGRYVPFHIQVPQKFFAIKNLLLLPGSYTYEWNFRKDVNMVLQSSLGNDLRVDGASIKFDSICLYATFFPMAHNTASTLEAMLRNDTNDQSFNDYLSAANMLYPIPANATNVPISIPSRNWAAFRGWAFTRLKTKETPSLGSGYDPYYTYSGSIPYLDGTFYLNHTFKKVAITFDSSVSWPGNDRLLTPNEFEIKRSVDGEGYNVAQCNMTKDWFLVQMLANYNIGYQGFYIPESYKDRMYSFFRNFQPMSRQVVDDTKYKDYQQVGILHQHNNSGFVGYLAPTMREGQAYPANFPYPLIGKTAVDSITQKKFLCDRTLWRIPFSSNFMSMGALTDLGQNLLYANSAHALDMTFEVDPMDEPTLLYVLFEVFDVVRVHQPHRGVIETVYLRTPFSAGNATT

SEQ ID NO: 6 - protein, 13 aa, Human Adenovirus Species C
EEEDDDNEDEVDE

SEQ ID NO: 7 - protein, 38 aa, Human Adenovirus Species C
EQEEPTQEMAEELEDEEEAEEEEAEEEAEAPQADQKVK

SEQ ID NO: 8 - protein, 36 aa, Human Adenovirus Species C
EQTEDSGRAVAEDEEEEDEDEEEEEEEQNARDQATK

SEQ ID NO: 9 - protein, 32 aa, Human Adenovirus Species C
EQNETAQVDAQELDEEENEANEAQAREQEQAK

SEQ ID NO: 10 - protein, 31 aa, Human Adenovirus Species C
DEDDTQVQVAAEDDQDDDEEEEQLPQQRNGK

SEQ ID NO: 11 - protein, 946 aa, Human Adenovirus Species C
MATPSMMPQWSYMHISGQDASEYLSPGLVQFARATETYFSLNNKFRNPTVAPTHDVTTDRSQRLTLRFIPVDREDTAYSYKARFTLAVGDNRVLDMASTYFDIRGVLDRGPTFKPYSGTAYNALAPKGAPNSCEWDEAATALEINLKKKKQAEQQKTHVYAQAPLAGEKITANGLQIVSDTQTEGNPVFADPTYQPEPQVGESQWNEAEATASGGRVLKKTTPMKPCYGSYARPTNKNGGQGILVANNQGALESKVEMQFFAPSGTAMNERNAVQPSIVLYSEDVNMETPDTHISYKPSKTDENSKAMLGQQAMPNRPNYIAFRDNFIGLMYYNSTGNMGVLAGQASQLNAVVDLQDRNTELSYQLLLDSIGDRTRYFSMWNQAVDSYDPDVRIIENHGTEDELPNYCFPLGGIGVTDTYQGIKSNGNGNPQNWTKNDDFAARNEIGVGNNFALEINLNANLWRNFLYSNIALYLPDKLKYTPTNVEISPNPNSYDYMNKRVVAPGLVDCYINLGARWSLDYMDNVNPFNHHRNAGLRYRSMLLGNGRYVPFHIQVPQKFFAIKNLLLLPGSYTYEWNFRKDVNMVLQSSLGNDLRVDGASIKFDSICLYATFFPMAHNTASTLEAMLRNDTNDQSFNDYLSAANMLYPIPANATNVPISIPSRNWAAFRGWAFTRLKTKETPSLGSGYDPYYTYSGSIPYLDGTFYLNHTFKKVAITFDSSVSWPGNDRLLTPNEFEIKRSVDGEGYNVAQCNMTKDWFLVQMLANYNIGYQGFYIPESYKDRMYSFFRNFQPMSRQVVDDTKYKDYQQVGILHQHNNSGFVGYLAPTMREGQAYPANFPYPLIGKTAVDSITQKKFLCDRTLWRIPFSSNFMSMGALTDLGQNLLYANSAHALDMTFEVDPMDEPTLLYVLFEVFDVVRVHQPHRGVIETVYLRTPFSAGNATT

SEQ ID NO: 12 - protein, 952 aa, Human Adenovirus Species C
MATPSMMPQWSYMHISGQDASEYLSPGLVQFARATETYFSLNNKFRNPTVAPTHDVTTDRSQRLTLRFIPVDREDTAYSYKARFTLAVGDNRVLDMASTYFDIRGVLDRGPTFKPYSGTAYNALAPKGAPNSCEWDEAATALEINLKKKKQAEQQKTHVYAQAPLSGETITKSGLQIGSDNAETQTKPVYADPSYQPEPQIGESQWNEADANAAGGRVLKKTTPMKPCYGSYARPTNPFGGQSVLVPDEKGVPLPKVDLQFFSNTTSLNDRQGNATKPKVVLYSEDVNMETPDTHLSYKPGKGDENSKAMLGQQSMPNRPNYIAFRDNFIGLMYYNSTGNMGVLAGQASQLNAVVDLQDRNTELSYQLLLDSIGDRTRYFSMWNQAVDSYDPDVRIIENHGTEDELPNYCFPLGGIGVTDTYQAIKANGNGSGDNGDTTWTKDETFATRNEIGVGNNFAMEINLNANLWRNFLYSNIALYLPDKLKYNPTNVEISDNPNTYDYMNKRVVAPGLVDCYINLGARWSLDYMDNVNPFNHHRNAGLRYRSMLLGNGRYVPFHIQVPQKFFAIKNLLLLPGSYTYEWNFRKDVNMVLQSSLGNDLRVDGASIKFDSICLYATFFPMAHNTASTLEAMLRNDTNDQSFNDYLSAANMLYPIPANATNVPISIPSRNWAAFRGWAFTRLKTKETPSLGSGYDPYYTYSGSIPYLDGTFYLNHTFKKVAITFDSSVSWPGNDRLLTPNEFEIKRSVDGEGYNVAQCNMTKDWFLVQMLANYNIGYQGFYIPESYKDRMYSFFRNFQPMSRQVVDDTKYKEYQQVGILHQHNNSGFVGYLAPTMREGQAYPANVPYPLIGKTAVDSITQKKFLCDRTLWRIPFSSNFMSMGALTDLGQNLLYANSAHALDMTFEVDPMDEPTLLYVLFEVFDVVRVHQPHRGVIETVYLRTPFSAGNATT

SEQ ID NO: 13 - protein, 951 aa, Human Adenovirus Species C
MATPSMMPQWSYMHISGQDASEYLSPGLVQFARATETYFSLNNKFRNPTVAPTHDVTTDRSQRLTLRFIPVDREDTAYSYKARFTLAVGDNRVLDMASTYFDIRGVLDRGPTFKPYSGTAYNALAPKGAPNSCEWDEAATALEINLKKKKQAEQQKTHVYAQAPLSGIKITKEGLQIGTADATVAGAGKEIFADKTFQPEPQVGESQWNEADATAAGGRVLKKTTPMKPCYGSYARPTNSNGGQGVMVEQNGKLESQVEMQFFSTSTNATNEVNNIQPTVVLYSEDVNMETPDTHLSYKPKMGDKNAKVMLGQQAMPNRPNYIAFRDNFIGLMYYNSTGNMGVLAGQASQLNAVVDLQDRNTELSYQLLLDSIGDRTRYFSMWNQAVDSYDPDVRIIENHGTEDELPNYCFPLGGIGITDTFQAVKTTAANGDQGNTTWQKDSTFAERNEIGVGNNFAMEINLNANLWRNFLYSNIALYLPDKLKYNPTNVEISDNPNTYDYMNKRVVAPGLVDCYINLGARWSLDYMDNVNPFNHHRNAGLRYRSMLLGNGRYVPFHIQVPQKFFAIKNLLLLPGSYTYEWNFRKDVNMVLQSSLGNDLRVDGASIKFDSICLYATFFPMAHNTASTLEAMLRNDTNDQSFNDYLSAANMLYPIPANATNVPISIPSRNWAAFRGWAFTRLKTKETPSLGSGYDPYYTYSGSIPYLDGTFYLNHTFKKVAITFDSSVSWPGNDRLLTPNEFEIKRSVDGEGYNVAQCNMTKDWFLVQMLANYNIGYQGFYIPESYKDRMYSFFRNFQPMSRQVVDDTKYKDYQQVGIIHQHNNSGFVGYLAPTMREGQAYPANVPYPLIGKTAVDSITQKKFLCDRTLWRIPFSSNFMSMGALTDLGQNLLYANSAHALDMTFEVDPMDEPTLLYVLFEVFDVVRVHQPHRGVIETVYLRTPFSAGNATT

SEQ ID NO: 14 - protein, 948 aa, Human Adenovirus Species C
MATPSMMPQWSYMHISGQDASEYLSPGLVQFARATETYFSLNNKFRNPTVAPTHDVTTDRSQRLTLRFIPVDREDTAYSYKARFTLAVGDNRVLDMASTYFDIRGVLDRGPTFKPYSGTAYNALAPKGAPNSCEWDEAATALEINLKKKKQAEQQKTHVYAQAPFAGEAINKNGLQIGTNGAATEGNKEIYADKTYQPEPQIGESQWNEAESSVAGGRVLKKTTPMKPCYGSYARPTNSNGGQGVMVEQNGKLESQVEMQFFSTSVNAMNEANAIQPKLVLYSEDVNMETPDTHLSYKPGKSDDNSKAMLGQQSMPNRPNYIAFRDNFIGLMYYNSTGNMGVLAGQASQLNAVVDLQDRNTELSYQLLLDSIGDRTRYFSMWNQAVDSYDPDVRIIENHGTEDELPNYCFPLGGIGVTDTYQAIKATNGNGGATTWAQDNTFAERNEIGVGNNFAMEINLNANLWRNFLYSNIALYLPDKLKYNPTNVEISDNPNTYDYMNKRVVAPGLVDCYINLGARWSLDYMDNVNPFNHHRNAGLRYRSMLLGNGRYVPFHIQVPQKFFAIKNLLLLPGSYTYEWNFRKDVNMVLQSSLGNDLRVDGASIKFDSICLYATFFPMAHNTASTLEAMLRNDTNDQSFNDYLSAANMLYPIPANATNVPISIPSRNWAAFRGWAFTRLKTKETPSLGSGYDPYYTYSGSIPYLDGTFYLNHTFKKVAITFDSSVSWPGNDRLLTPNEFEIKRSVDGEGYNVAQCNMTKDWFLVQMLANYNIGYQGFYIPESYKDRMYSFFRNFQPMSRQVVDDTKYKDYQQVGILHQHNNSGFVGYLAPTMREGQAYPANFPYPLIGKTAVDSITQKKFLCDRTLWRIPFSSNFMSMGALTDLGQNLLYANSAHALDMTFEVDPMDEPTLLYVLFEVFDVVRVHQPHRGVIETVYLRTPFSAGNATT

SEQ ID NO: 15 - protein, 4 aa, Human Adenovirus Species C
KKKK

SEQ ID NO: 16 - protein, 13 aa, Human Adenovirus Species C
EEEKKKNEKEVDE

SEQ ID NO: 17 - protein, 20 aa, Human Adenovirus Species C
EINLEEEDDDNEDEVDEQAE

SEQ ID NO: 18 - protein, 13 aa, Human Adenovirus Species C
KINLKKNKVKQAK

SEQ ID NO: 19 - protein, 16 aa, Human Adenovirus Species C
STTEAAAGNGDNLTPK

SEQ ID NO: 20 - protein, 16 aa, Human Adenovirus Species C
STTKAAAGNGKNLTPK

SEQ ID NO: 21 - protein, 41 aa, Human Adenovirus Species C
GGVINTETLTKVKPKTGQENGWEKDATEFSDKNEIRVGNNF

SEQ ID NO: 22 - protein, 41 aa, Human Adenovirus Species C
GGVINTETLTKVKPKTGQKNGWKKKATEFSDKNEIRVGNNF

SEQ ID NO: 23 - DNA, 74 bp, Human Adenovirus Species C
caaatccttgcgaatgggatgaagctgctactgctcttgaaataaacctaggcctggtgatgatggcgggatcg

SEQ ID NO: 24 - DNA, 74 bp, Human Adenovirus Species C
ccagaataaggcgcctgcccaaatacgtgagttttttgctgctcagcttgtcagaagaactcgtcaagaaggcg

SEQ ID NO: 25 - DNA, 76 bp, Human Adenovirus Species C
ggagggcaaggcattcttgtaaagcaacaaaatggaaagctagaaagtcaagggcctggtgatgatggcgggatcg

SEQ ID NO: 26 - DNA, 76 bp, Human Adenovirus Species C
gtctggggtttctatatctacatcttcactgtacaataccactttaggagtctcagaagaactcgtcaagaaggcg

SEQ ID NO: 27 - DNA, 75 bp, Human Adenovirus Species C
catggaactgaagatgaacttccaaattactgctttccactgggaggtgtgggcctggtgatgatggcgggatcg

SEQ ID NO: 28 - DNA, 76 bp, Human Adenovirus Species C
ctccacaggttggcatttagattgatttccatggcaaaattatttccaactctcagaagaactcgtcaagaaggcg

SEQ ID NO: 29 - DNA, 24 bp, Human Adenovirus Species C
ttttaagccctactctggcactgc

SEQ ID NO: 30 - DNA, 24 bp, Human Adenovirus Species C
ccttcgacacctatttgaataccc

SEQ ID NO: 31 - DNA, 24 bp, Human Adenovirus Species C
cacaaatgaaaatggagggcaagg

SEQ ID NO: 32 - DNA, 24 bp, Human Adenovirus Species C
gtgggcatgtaagaaatatgagtg

SEQ ID NO: 33 - DNA, 25 bp, Human Adenovirus Species C
gacagctatgatccagatgttagaa

SEQ ID NO: 34 - DNA, 24 bp, Human Adenovirus Species C
ctccacaggttggcatttagattg

SEQ ID NO: 35 - DNA, 24 bp, Mus musculus
ctccacaggttggcatttagattg

SEQ ID NO: 36 - DNA, 24 bp, Mus musculus
ctccacaggttggcatttagattg

SEQ ID NO: 37 - DNA, 20 bp, Human Adenovirus Species C
tagacgatccctactgtacg

SEQ ID NO: 38 - DNA, 20 bp, Human Adenovirus Species C
ccggacgtagtcatatttcc

SEQ ID NO: 39 - DNA, 20 bp, Human Adenovirus Species C
ggaaatatgactacgtccgg

SEQ ID NO: 40 - DNA, 18 bp, Human Adenovirus Species C
gctcctcctgagcgcaag

SEQ ID NO: 41 - DNA, 20 bp, Human Adenovirus Species C
catctgctggaaggtggaca

SEQ ID NO: 42 - protein, 34 aa, Human Adenovirus Species C
DEAATALEINLEEEDDDNEDEVDEQAEQQKTHVF

SEQ ID NO: 43 - protein, 25 aa, Human Adenovirus Species C
DEAATALEINLKKKKQAEQQKTHVF

SEQ ID NO: 44 - DNA, 102 bp, Human Adenovirus Species C
gatgaagctgctactgctcttgaaataaacctagaagaagaggacgatgacaacgaagacgaagtagacgagcaagctgagcagcaaaaaactcacgtattt

SEQ ID NO: 45 - DNA, 75 bp, Human Adenovirus Species C
gatgaagctgctactgctcttgaaataaacctaaaaaagaaaaagcaagctgagcagcaaaaaactcacgtattt

SEQ ID NO: 46 - protein, 21 aa, Human Adenovirus Species C
DEAATALEINLQAEQQKTHVF

SEQ ID NO: 47 - protein, 34 aa, Human Adenovirus Species C
DEAATALEINLEEEKKKNEKEVDEQAEQQKTHVF

SEQ ID NO: 48 - protein, 27 aa, Human Adenovirus Species C
DEAATALKINLKKNKVKQAKQQKTHVF

SEQ ID NO: 49 - protein, 37 aa, Human Adenovirus Species C
EQTEDSGRAVAEDEEEEEDEDEEEEEEEQNARDQATK

SEQ ID NO: 50 - protein, 952 aa, Human Adenovirus Species C
MATPSMMPQWSYMHISGQDASEYLSPGLVQFARATETYFSLNNKFRNPTVAPTHDVTTDRSQRLTLRFIPVDREDTAYSYKARFTLAVGDNRVLDMASTYFDIRGVLDRGPTFKPYSGTAYNALAPKGAPNSCEWDEAATALEINLKKKKQAEQQKTHVYAQAPLSGETITKSGLQIGSDNAETQAKPVYADPSYQPEPQIGESQWNEADANAAGGRVLKKTTPMKPCYGSYARPTNPFGGQSVLVPDEKGVPLPKVDLQFFSNTTSLNDRQGNATKPKVVLYSEDVNLETPDTHLSYKPGKGDENSKAMLGQQSMPNRPNYIAFRDNFIGLMYYNSTGNMGVLAGQASQLNAVVDLQDRNTELSYQLLLDSIGDRTRYFSMWNQAVDSYDPDVRIIENHGTEDELPNYCFPLGGIGVTDTYQAIKANGNGAGDNGNTTWTKDETFATRNEIGVGNNFAMEINLNANLWRNFLYSNIALYLPDKLKYNPTNVEISDNPNTYDYMNKRVVAPGLVDCYINLGARWSLDYMDNVNPFNHHRNAGLRYRSMLLGNGRYVPFHIQVPQKFFAIKNLLLLPGSYTYEWNFRKDVNMVLQSSLGNDLRVDGASIKFDSICLYATFFPMAHNTASTLEAMLRNDTNDQSFNDYLSAANMLYPIPANATNVPISIPSRNWAAFRGWAFTRLKTKETPSLGSGYDPYYTYSGSIPYLDGTFYLNHTFKKVAITFDSSVSWPGNDRLLTPNEFEIKRSVDGEGYNVAQCNMTKDWFLVQMLANYNIGYQGFYIPESYKDRMYSFFRNFQPMSRQVVDDTKYKDYQQVGIIHQHNNSGFVGYLAPTMREGQAYPANVPYPLIGKTAVDSITQKKFLCDRTLWRIPFSSNFMSMGALTDLGQNLLYANSAHALDMTFEVDPMDEPTLLYVLFEVFDVVRVHQPHRGVIETVYLRTPFSAGNATT

SEQ ID NO: 51 - protein, 27 aa, Human Adenovirus Species C
DEAATALEINLKKKKKKQAEQQKTHVF

SEQ ID NO: 52 - protein, 29 aa, Human Adenovirus Species C
DEAATALEINLKKKKKKKKQAEQQKTHVF

SEQ ID NO: 53 - protein, 45 aa, Human Adenovirus Species C
DEAATALEINLGGSGGGSGKKKKKKKKGSGGGSGGQAEQQKTHVF